European Patent Specification EP 4 083 207 B1, published March 25, 2026. Title: Method for inhibiting methylation of target DNA in plant. Applicant: National Institute of Advanced Industrial Science and Technology et al. Application JP 2019-237374. The sequence listing filed with the application follows.

SEQUENCE LISTING (8 sequences)

SEQ ID NO: 1 - DNA, 345 bp, Cauliflower mosaic virus
tctctccaaatgaaatgaacttccttatatagaggaagggtcttgcgaaggatagtgggattgtgcgtcatcccttacgtcagtggagatatcacatcaatccacttgctttgaagacgtggttggaacgtcttctttttccacgatgctcctcgtgggtgggggtccatctttgggaccactgtcggcagaggcatcttcaacgatggcctttcctttatcgcaatgatggcatttgtaggagccaccttccttttccactatcttcacaataaagtgacagatagctgggcaatggaatccgaggaggtttccggatattaccctttgttgaaaagtctcaat

SEQ ID NO: 2 - DNA, 26 bp, Artificial Sequence
  Short dummy RNA_SD-51
taagggaggacgcacaatccccctat

SEQ ID NO: 3 - DNA, 33 bp, Artificial Sequence
  35S(-)-sdRNA-(-51)-5St
cgaggccttaagggatgacgcacaatcccacta

SEQ ID NO: 4 - DNA, 35 bp, Artificial Sequence
  35S(-)-sdRNA-(-51)-3Ml
cgcacgcgtatagtgggattgtgcgtcatccctta

SEQ ID NO: 5 - DNA, 24 bp, Artificial Sequence
  35S-346F-bisuT
attgagayttttyaayaaagggta

SEQ ID NO: 6 - DNA, 22 bp, Artificial Sequence
  35S+1A-bisuA
ctctccaaatgaaatgaacttc

SEQ ID NO: 7 - DNA, 26 bp, Artificial Sequence
  35S(-)-5-BS
ttatatagaggaagggtyttgygaag

SEQ ID NO: 8 - DNA, 22 bp, Artificial Sequence
  35S(-)-3-BS
caattraracttttcaacaaar